European Patent Specification EP 3 708 579 B1, published May 1, 2024. Title: CLAUDIN-6-SPECIFIC IMMUNORECEPTORS AND T CELL EPITOPES. Applicant: BioNTech Cell & Gene Therapies GmbH et al. The sequence listing filed with the application follows.

SEQUENCE LISTING (46 sequences)

SEQ ID NO: 1 - protein, 220 aa, Homo sapiens
MASAGMQILGVVLTLLGWVNGLVSCALPMWKVTAFIGNSIVVAQVVWEGLWMSCVVQSTGQMQCKVYDSLLALPQDLQAARALCVIALLVALFGLLVYLAGAKCTTCVEEKDSKARLVLTSGIVFVISGVLTLIPVCWTAHAIIRDFYNPLVAEAQKRELGASLYLGWAASGLLLLGGGLLCCTCPSGGSQGPSHYMARYSTSAPAISRGPSEYPTKNYV

SEQ ID NO: 2 - protein, 220 aa, Homo sapiens
MASAGMQILGVVLTLLGWVNGLVSCALPMWKVTAFIGNSIVVAQVVWEGLWMSCVVQSTGQMQCKVYDSLLALPQDLQAARALCVIALLVALFGLLVYLAGAKCTTCVEEKDSKARLVLTSGIVFVISGVLTLIPVCWTAHAVIRDFYNPLVAEAQKRELGASLYLGWAASGLLLLGGGLLCCTCPSGGSQGPSHYMARYSTSAPAISRGPSEYPTKNYV

SEQ ID NO: 3 - protein, 9 aa, Artificial Sequence
  T cell epitope
ALFGLLVYL

SEQ ID NO: 4 - protein, 9 aa, Artificial Sequence
  T cell epitope
TLLGWVNGL

SEQ ID NO: 5 - protein, 9 aa, Artificial Sequence
  T cell epitope
QILGVVLTL

SEQ ID NO: 6 - protein, 269 aa, Homo sapiens
MLLALLSVLGIHFLLRDAQAQSVTQPDARVTVSEGASLQLRCKYSYFGTPYLFWYVQYPRQGLQLLLKYYPGDPVVQGVNGFEAEFSKSNSSFHLRKASVHWSDWAVYFCAVSMSSGTYQRFGTGTKLQVVPNIQNPEPAVYQLKDPRSQDSTLCLFTDFDSQINVPKTMESGTFITDKTVLDMKAMDSKSNGAIAWSNQTSFTCQDIFKETNATYPSSDVPCDATLTEKSFETDMNLNFQNLSVMGLRILLLKVAGFNLLMTLRLWSS

SEQ ID NO: 7 - protein, 304 aa, Homo sapiens
MRVRLISAVVLCFLGTGLVDMKVTQMPRYLIKRMGENVLLECGQDMSHETMYWYRQDPGLGLQLIYISYDVDSNSEGDIPKGYRVSRKKREHFSLILDSAKTNQTSVYFCASSSQNQDTQYFGPGTRLLVLEDLRNVTPPKVSLFEPSKAEIANKQKATLVCLARGFFPDHVELSWWVNGKEVHSGVSTDPQAYKESNYSYCLSSRLRVSATFWHNPRNHFRCQVQFHGLSEEDKWPEGSPKPVTQNISAEAWGRADCGITSASYHQGVLSATILYEILLGKATLYAVLVSGLVLMAMVKKKNS

SEQ ID NO: 8 - protein, 268 aa, Homo sapiens
MDSFPGFVAVILLILGRTHGDSVTQTEGQVTVSESKSLIINCTYSATSIGYPNLFWYVRYPGEGLQLLLKVITAGQKGSSRGFEATYNKEATSFHLQKASVQESDSAVYYCALNNQGKLIFGQGTKLSIKPNIQNPEPAVYQLKDPRSQDSTLCLFTDFDSQINVPKTMESGTFITDKTVLDMKAMDSKSNGAIAWSNQTSFTCQDIFKETNATYPSSDVPCDATLTEKSFETDMNLNFQNLSVMGLRILLLKVAGFNLLMTLRLWSS

SEQ ID NO: 9 - protein, 303 aa, Homo sapiens
MGSRLFFVLSSLLCSKHMEAAVTQSPRNKVAVTGGKVTLSCNQTNNHNNMYWYRQDTGHGLRLIHYSYGAGSTEKGDIPDGYKASRPSQENFSLILELATPSQTSVYFCASGGDSQNTLYFGAGTRLSVLEDLRNVTPPKVSLFEPSKAEIANKQKATLVCLARGFFPDHVELSWWVNGKEVHSGVSTDPQAYKESNYSYCLSSRLRVSATFWHNPRNHFRCQVQFHGLSEEDKWPEGSPKPVTQNISAEAWGRADCGITSASYHQGVLSATILYEILLGKATLYAVLVSGLVLMAMVKKKNS

SEQ ID NO: 10 - protein, 273 aa, Homo sapiens
MLILSLLGAAFGSICFATSMAQKVTQTQTSISVVEKTTVTMDCVYETRDSSYFLFWYKQTASGEIVFLIRQDSYKKENATVGHYSLNFQKPKSSIGLIITATQIEDSAVYFCAMREAANSGTYQRFGTGTKLQVVPNIQNPEPAVYQLKDPRSQDSTLCLFTDFDSQINVPKTMESGTFITDKTVLDMKAMDSKSNGAIAWSNQTSFTCQDIFKETNATYPSSDVPCDATLTEKSFETDMNLNFQNLSVMGLRILLLKVAGFNLLMTLRLWSS

SEQ ID NO: 11 - protein, 305 aa, Homo sapiens
MGSIFLSCLAVCLLVAGPVDPKIIQKPKYLVAVTGSEKILICEQYLGHNAMYWYRQSAKKPLEFMFSYSYQKLMDNQTASSRFQPQSSKKNHLDLQITALKPDDSATYFCASSQQNSGNTLYFGEGSRLIVVEDLRNVTPPKVSLFEPSKAEIANKQKATLVCLARGFFPDHVELSWWVNGKEVHSGVSTDPQAYKESNYSYCLSSRLRVSATFWHNPRNHFRCQVQFHGLSEEDKWPEGSPKPVTQNISAEAWGRADCGITSASYQQGVLSATILYEILLGKATLYAVLVSTLVVMAMVKRKNS

SEQ ID NO: 12 - protein, 270 aa, Homo sapiens
MKTVTGPLFLCFWLQLNCVSRGEQVEQRPPHLSVREGDSAVITCTYTDPNSYYFFWYKQEPGASLQLLMKVFSSTEINEGQGFTVLLNKKDKRLSLNLTAAHPGDSAAYFCAVESSSFSKLVFGQGTSLSVVPNIQNPEPAVYQLKDPRSQDSTLCLFTDFDSQINVPKTMESGTFITDKTVLDMKAMDSKSNGAIAWSNQTSFTCQDIFKETNATYPSSDVPCDATLTEKSFETDMNLNFQNLSVMGLRILLLKVAGFNLLMTLRLWSS

SEQ ID NO: 13 - protein, 307 aa, Homo sapiens
MATRLLCYTVLCLLGARILNSKVIQTPRYLVKGQGQKAKMRCIPEKGHPVVFWYQQNKNNEFKFLINFQNQEVLQQIDMTEKRFSAECPSNSPCSLEIQSSEAGDSALYLCASSLTGGAQDTQYFGPGTRLLVLEDLRNVTPPKVSLFEPSKAEIANKQKATLVCLARGFFPDHVELSWWVNGKEVHSGVSTDPQAYKESNYSYCLSSRLRVSATFWHNPRNHFRCQVQFHGLSEEDKWPEGSPKPVTQNISAEAWGRADCGITSASYHQGVLSATILYEILLGKATLYAVLVSGLVLMAMVKKKNS

SEQ ID NO: 14 - protein, 266 aa, Homo sapiens
MQRNLVAVLGILWVQICWVRGDQVEQSPSALSLHEGTGSALRCNFTTTMRAVQWFRKNSRGSLINLFYLASGTKENGRLKSAFDSKERYSTLHIRDAQLEDSGTYFCAAEGGGNYKPTFGKGTSLVVHPYIQNPEPAVYQLKDPRSQDSTLCLFTDFDSQINVPKTMESGTFITDKTVLDMKAMDSKSNGAIAWSNQTSFTCQDIFKETNATYPSSDVPCDATLTEKSFETDMNLNFQNLSVMGLRILLLKVAGFNLLMTLRLWSS

SEQ ID NO: 15 - protein, 302 aa, Homo sapiens
MLYSLLAFLLGMFLGVSAQTIHQWPVAEIKAVGSPLSLGCTIKGKSSPNLYWYWQATGGTLQQLFYSITVGQVESVVQLNLSASRPKDDQFILSTEKLLLSHSGFYLCAWSPPINTEVFFGKGTRLTVVEDLRNVTPPKVSLFEPSKAEIANKQKATLVCLARGFFPDHVELSWWVNGKEVHSGVSTDPQAYKESNYSYCLSSRLRVSATFWHNPRNHFRCQVQFHGLSEEDKWPEGSPKPVTQNISAEAWGRADCGITSASYQQGVLSATILYEILLGKATLYAVLVSTLVVMAMVKRKNS

SEQ ID NO: 16 - protein, 271 aa, Homo sapiens
MDSSPGFVAVILLILGRTHGDSVTQTEGPVTVSESESLIINCTYSATSIAYPNLFWYVRYPGEGLQLLLKVITAGQKGSSRGFEATYNKETTSFHLQKASVQESDSAVYYCALGETGSFNKLTFGAGTRLAVCPYIQNPEPAVYQLKDPRSQDSTLCLFTDFDSQINVPKTMESGTFITDKTVLDMKAMDSKSNGAIAWSNQTSFTCQDIFKETNATYPSSDVPCDATLTEKSFETDMNLNFQNLSVMGLRILLLKVAGFNLLMTLRLWSS

SEQ ID NO: 17 - protein, 304 aa, Homo sapiens
MATRLLCYTVLCLLGARILNSKVIQTPRYLVKGQGQKAKMRCIPEKGHPVVFWYQQNKNNEFKFLINFQNQEVLQQIDMTEKRFSAECPSNSPCSLEIQSSEAGDSALYLCASSLGIYEQYFGPGTRLTVLEDLRNVTPPKVSLFEPSKAEIANKQKATLVCLARGFFPDHVELSWWVNGKEVHSGVSTDPQAYKESNYSYCLSSRLRVSATFWHNPRNHFRCQVQFHGLSEEDKWPEGSPKPVTQNISAEAWGRADCGITSASYHQGVLSATILYEILLGKATLYAVLVSGLVLMAMVKKKNS

SEQ ID NO: 18 - protein, 274 aa, Homo sapiens
MLILSLLGAAFGSICFAATSMAQKVTQTQTSISVVEKTTVTMDCVYETRDSSYFLFWYKQTASGEIVFLIRQDSYKKENATVGHYSLNFQKPKSSIGLIITATQIEDSAVYFCAMRDSSGGNYKPTFGKGTSLVVHPYIQNPEPAVYQLKDPRSQDSTLCLFTDFDSQINVPKTMESGTFITDKTVLDMKAMDSKSNGAIAWSNQTSFTCQDIFKETNATYPSSDVPCDATLTEKSFETDMNLNFQNLSVMGLRILLLKVAGFNLLMTLRLWSS

SEQ ID NO: 19 - protein, 307 aa, Homo sapiens
MGSIFLSCLAVCLLVAGPVDPKIIQKPKYLVAVTGSEKILICEQYLGHNAMYWYRQSAKKPLEFMFSYSYQKLMDNQTASSRFQPQSSKKNHLDLQITALKPDDSATYFCASSQEDWGSQNTLYFGAGTRLSVLEDLRNVTPPKVSLFEPSKAEIANKQKATLVCLARGFFPDHVELSWWVNGKEVHSGVSTDPQAYKESNYSYCLSSRLRVSATFWHNPRNHFRCQVQFHGLSEEDKWPEGSPKPVTQNISAEAWGRADCGITSASYHQGVLSATILYEILLGKATLYAVLVSGLVLMAMVKKKNS

SEQ ID NO: 20 - protein, 269 aa, Homo sapiens
MKRLVCSLLGLLCTQVCWVKGQQVQQSPASLVLQEGENAELQCNFSSTATRLQWFYQRPGGSLVSLLYNPSGTKHTGRLTSTTVTKERRSSLHISSSQTTDSGTYFCAMSSNSGGSNAKLTFGKGTKLSVKSNIQNPEPAVYQLKDPRSQDSTLCLFTDFDSQINVPKTMESGTFITDKTVLDMKAMDSKSNGAIAWSNQTSFTCQDIFKETNATYPSSDVPCDATLTEKSFETDMNLNFQNLSVMGLRILLLKVAGFNLLMTLRLWSS

SEQ ID NO: 21 - protein, 305 aa, Homo sapiens
MGCRLLSCVAFCLLGIGPLETAVFQTPNYRVTRVGNEVSFNCEQTLDHNTMYWYKQDSKKLLKIMFSYNNKQLIVNETVPRRFSPQSSDKAHLNLRIKSVELEDSAVYLCASSDWGDSYEQYFGPGTRLTVLEDLRNVTPPKVSLFEPSKAEIANKQKATLVCLARGFFPDHVELSWWVNGKEVHSGVSTDPQAYKESNYSYCLSSRLRVSATFWHNPRNHFRCQVQFHGLSEEDKWPEGSPKPVTQNISAEAWGRADCGITSASYHQGVLSATILYEILLGKATLYAVLVSGLVLMAMVKKKNS

SEQ ID NO: 22 - protein, 274 aa, Homo sapiens
MLILSLLGAAFGSICFAATSMAQKVTQTQTSISVVEKTTVTMDCVYETRDSSYFLFWYKQTASGEIVFLIRQDSYKKENATVGHYSLNFQKPKSSIGLIITATQIEDSAVYFCAMRVASSGSWQLIFGSGTQLTVMPDIQNPEPAVYQLKDPRSQDSTLCLFTDFDSQINVPKTMESGTFITDKTVLDMKAMDSKSNGAIAWSNQTSFTCQDIFKETNATYPSSDVPCDATLTEKSFETDMNLNFQNLSVMGLRILLLKVAGFNLLMTLRLWSS

SEQ ID NO: 23 - protein, 306 aa, Homo sapiens
MGSIFLSCLAVCLLVAGPVDPKIIQKPKYLVAVTGSEKILICEQYLGHNAMYWYRQSAKKPLEFMFSYSYQKLMDNQTASSRFQPQSSKKNHLDLQITALKPDDSATYFCASSQGDNNYAEQFFGPGTRLTVLEDLRNVTPPKVSLFEPSKAEIANKQKATLVCLARGFFPDHVELSWWVNGKEVHSGVSTDPQAYKESNYSYCLSSRLRVSATFWHNPRNHFRCQVQFHGLSEEDKWPEGSPKPVTQNISAEAWGRADCGITSASYHQGVLSATILYEILLGKATLYAVLVSGLVLMAMVKKKNS

SEQ ID NO: 24 - protein, 268 aa, Homo sapiens
MKTVTGPLLLCFWLQLNCVSRGEQVEQRPPHLSVREGDSAIIICTYTDSATAYFSWYKQEAGAGLQLLMSVLSNVDRKEEQGLTVLLNKKDKRLSLNLTAAHPGDSAVYFCATNAGAKLTFGGGTRLTVRPDIQNPEPAVYQLKDPRSQDSTLCLFTDFDSQINVPKTMESGTFITDKTVLDMKAMDSKSNGAIAWSNQTSFTCQDIFKETNATYPSSDVPCDATLTEKSFETDMNLNFQNLSVMGLRILLLKVAGFNLLMTLRLWSS

SEQ ID NO: 25 - protein, 306 aa, Homo sapiens
MGCRLLSCVAFCLLGIGPLETAVFQTPNYHVTQVGNEVSFNCKQTLGHDTMYWYKQDSKKLLKIMFSYNNKQLIVNETVPRRFSPQSSDKAHLNLRIKSVEPEDSAVYLCASSLYWGDSYEQYFGPGTRLTVLEDLRNVTPPKVSLFEPSKAEIANKQKATLVCLARGFFPDHVELSWWVNGKEVHSGVSTDPQAYKESNYSYCLSSRLRVSATFWHNPRNHFRCQVQFHGLSEEDKWPEGSPKPVTQNISAEAWGRADCGITSASYHQGVLSATILYEILLGKATLYAVLVSGLVLMAMVKKKNS

SEQ ID NO: 26 - protein, 277 aa, Homo sapiens
MDKNLTASFLLLGLHLAGVSGQQEKRDQQQVRQSPQSLTVWEGETAILNCSYENSAFDYFPWYQQFPGEGPALLISILSVSDKKEDGRFTIFFNKREKKLSLHIADSQPGDSATYFCAASLSSGSWQLIFGSGTQLTVMPDIQNPEPAVYQLKDPRSQDSTLCLFTDFDSQINVPKTMESGTFITDKTVLDMKAMDSKSNGAIAWSNQTSFTCQDIFKETNATYPSSDVPCDATLTEKSFETDMNLNFQNLSVMGLRILLLKVAGFNLLMTLRLWSS

SEQ ID NO: 27 - protein, 305 aa, Homo sapiens
MDIWLLGWIIFSFLEAGHTGPKVLQIPSHQIIDMGQMVTLNCDPVSNHLYFYWYKQILGQQMEFLVNFYNGKVMEKSKLFKDQFSVERPDGSYFTLKIQPTALEDSAVYFCASSLVGGYEQYFGPGTRLTVLEDLRNVTPPKVSLFEPSKAEIANKQKATLVCLARGFFPDHVELSWWVNGKEVHSGVSTDPQAYKESNYSYCLSSRLRVSATFWHNPRNHFRCQVQFHGLSEEDKWPEGSPKPVTQNISAEAWGRADCGITSASYHQGVLSATILYEILLGKATLYAVLVSGLVLMAMVKKKNS

SEQ ID NO: 28 - protein, 268 aa, Homo sapiens
MDSFPGFMTVMLLIFTRAHGDSVTQTEGQVALSEEDFLTIHCNYSASGYPALFWYVQYPGEGPQFLFRASRDKEKGSSRGFEATYDKGTTSFHLRKASVQESDSAVYYCALGNNYAQGLTFGLGTRVSVFPYIQNPEPAVYQLKDPRSQDSTLCLFTDFDSQINVPKTMESGTFITDKTVLDMKAMDSKSNGAIAWSNQTSFTCQDIFKETNATYPSSDVPCDATLTEKSFETDMNLNFQNLSVMGLRILLLKVAGFNLLMTLRLWSS

SEQ ID NO: 29 - protein, 302 aa, Homo sapiens
MGSRLFFVVLILLCAKHMEAAVTQSPRSKVAVTGGKVTLSCHQTNNHDYMYWYRQDTGHGLRLIHYSYVADSTEKGDIPDGYKASRPSQENFSLILELASLSQTAVYFCASSTGNERLFFGHGTKLSVLEDLRNVTPPKVSLFEPSKAEIANKQKATLVCLARGFFPDHVELSWWVNGKEVHSGVSTDPQAYKESNYSYCLSSRLRVSATFWHNPRNHFRCQVQFHGLSEEDKWPEGSPKPVTQNISAEAWGRADCGITSASYQQGVLSATILYEILLGKATLYAVLVSTLVVMAMVKRKNS

SEQ ID NO: 30 - protein, 117 aa, Artificial Sequence
  Antibody fragment
EVQLQQSGPELVKPGASMKISCKASGYSFTGYTMNWVKQSHGKNLEWIGLINPYNGGTSYNQKFKGKATLTIDKSSSTAYMELLSLTSEDSAVYYCARDYGYVLDYWGQGTTLTVSS

SEQ ID NO: 31 - protein, 106 aa, Artificial Sequence
  Antibody fragment
IVLTQSPAIMSASPGEKVTITCSASSSVSYLHWFQQKPGTSPKLWVYSTSNLPSGVPARFGGSGSGTSYSLTISRMEAEDAATYYCQQRSIYPPWTFGGGTKLEIK

SEQ ID NO: 32 - protein, 117 aa, Artificial Sequence
  Antibody fragment
EVQLQQSGPELVKPGASMKISCKASGYSFTGYTMNWVKQSHGKNLEWIGLINPYNGGTIYNQKFKGKATLTVDKSSSTAYMELLSLTSEDSAVYYCARDYGFVLDYWGQGTTLTVSS

SEQ ID NO: 33 - protein, 106 aa, Artificial Sequence
  Antibody fragment
IVLTQSPSIMSVSPGEKVTITCSASSSVSYMHWFQQKPGTSPKLCIYSTSNLASGVPARFSGRGSGTSYSLTISRVAAEDAATYYCQQRSNYPPWTFGGGTKLEIK

SEQ ID NO: 34 - protein, 117 aa, Artificial Sequence
  Antibody fragment
EVQLQQSGPELVKPGASMKISCKASGYSFTGYTMNWVKQSHGKNLEWIGLINPYNGGIIYNQKFKGKATLTVDKSSSTAYMELLSLTSEDSAVFYCARDFGYVLDYWGQGTTLTVSS

SEQ ID NO: 35 - protein, 106 aa, Artificial Sequence
  Antibody fragment
IVLTQSPAIMSASPGEKVTITCSASSSVSYMHWFQQKPGTSPKLWIYSTSNLASGVPARFSGSGSGTSYSLTISRVAAEDAATYYCQQRSTYPPWTFGGGTKLEIK

SEQ ID NO: 36 - protein, 117 aa, Artificial Sequence
  Antibody fragment
EVQLQQSRPELVKPGASMKISCKASGYSFTGYTLNWVKQSHGKNLEWIGLINPYNGGSSYNQKFKDKATLTVDKSSSTAYMELLSLTSEDSAVYYCARDYGYVFDYWGQGTTLTVSS

SEQ ID NO: 37 - protein, 106 aa, Artificial Sequence
  Antibody fragment
IVLTQSPAIMSASPGEKVTITCSASSSVNYMHWFQLKPGTSPKLLIYSTSNLASGVPARFSGRGSGTSYSLTISRMEAEDAATYYCQQRNNYPPWTFGGGTKLEIK

SEQ ID NO: 38 - protein, 106 aa, Artificial Sequence
  Antibody fragment
IVLTQSPSIMSVSPGEKVTITCSASSSVSYMHWFQQKPGTSPKLGIYSTSNLASGVPARFSGRGSGTSYSLTISRVAAEDAATYYCQQRSNYPPWTFGGGTKLEIK

SEQ ID NO: 39 - protein, 106 aa, Artificial Sequence
  Antibody fragment
IVLTQSPSIMSVSPGEKVTITCSASSSVSYMHWFQQKPGTSPKLSIYSTSNLASGVPARFSGRGSGTSYSLTISRVAAEDAATYYCQQRSNYPPWTFGGGTKLEIK

SEQ ID NO: 40 - protein, 239 aa, Artificial Sequence
  mouse IgG VH-VL (kappa)
EVQLQQSGPELVKPGASMKISCKASGYSFTGYTMNWVKQSHGKNLEWIGLINPYNGGTIYNQKFKGKATLTVDKSSSTAYMELLSLTSEDSAVYYCARDYGFVLDYWGQGTTLTVSSGGGGSGGGGSGGGGSDIVLTQSPSIMSVSPGEKVTITCSASSSVSYMHWFQQKPGTSPKLSIYSTSNLASGVPARFSGRGSGTSYSLTISRVAAEDAATYYCQQRSNYPPWTFGGGTKLEIK

SEQ ID NO: 41 - protein, 15 aa, Artificial Sequence
  Linker
GGGGSGGGGSGGGGS

SEQ ID NO: 42 - protein, 19 aa, Artificial Sequence
  Signal peptide
MDWIWRILFLVGAATGAHS

SEQ ID NO: 43 - protein, 231 aa, Artificial Sequence
  human IgG1 Fc fragment
EPKSPDKTHTCPPCPAPPVAGPSVFLFPPKPKDTLMIARTPEVTCVVVDVSHEDPEVKFNWYVDGVEVHNAKTKPREEQYNSTYRVVSVLTVLHQDWLNGKEYKCKVSNKALPAPIEKTISKAKGQPREPQVYTLPPSRDELTKNQVSLTCLVKGFYPSDIAVEWESNGQPENNYKTTPPVLDSDGSFFLYSKLTVDKSRWQQGNVFSCSVMHEALHNHYTQKSLSLSPGK

SEQ ID NO: 44 - protein, 68 aa, Artificial Sequence
  human CD28 (TM + ic)
FWVLVVVGGVLACYSLLVTVAFIIFWVRSKRSRLLHSDYMNMTPRRPGPTRKHYQAYAAARDFAAYRS

SEQ ID NO: 45 - protein, 113 aa, Artificial Sequence
  human CD3-zeta (ic)
LRVKFSRSADAPAYQQGQNQLYNELNLGRREEYDVLDKRRGRDPEMGGKPRRKNPQEGLYNELQKDKMAEAYSEIGMKGERRRGKGHDGLYQGLSTATKDTYDALHMQALPPR

SEQ ID NO: 46 - protein, 679 aa, Artificial Sequence
  Artificial T cell receptor
MDWIWRILFLVGAATGAHSEVQLQQSGPELVKPGASMKISCKASGYSFTGYTMNWVKQSHGKNLEWIGLINPYNGGTIYNQKFKGKATLTVDKSSSTAYMELLSLTSEDSAVYYCARDYGFVLDYWGQGTTLTVSSGGGGSGGGGSGGGGSDIVLTQSPSIMSVSPGEKVTITCSASSSVSYMHWFQQKPGTSPKLSIYSTSNLASGVPARFSGRGSGTSYSLTISRVAAEDAATYYCQQRSNYPPWTFGGGTKLEIKRSDPAEPKSPDKTHTCPPCPAPPVAGPSVFLFPPKPKDTLMIARTPEVTCVVVDVSHEDPEVKFNWYVDGVEVHNAKTKPREEQYNSTYRVVSVLTVLHQDWLNGKEYKCKVSNKALPAPIEKTISKAKGQPREPQVYTLPPSRDELTKNQVSLTCLVKGFYPSDIAVEWESNGQPENNYKTTPPVLDSDGSFFLYSKLTVDKSRWQQGNVFSCSVMHEALHNHYTQKSLSLSPGKKDPKFWVLVVVGGVLACYSLLVTVAFIIFWVRSKRSRLLHSDYMNMTPRRPGPTRKHYQAYAAARDFAAYRSLRVKFSRSADAPAYQQGQNQLYNELNLGRREEYDVLDKRRGRDPEMGGKPRRKNPQEGLYNELQKDKMAEAYSEIGMKGERRRGKGHDGLYQGLSTATKDTYDALHMQALPPR